European Patent Application EP 4 652 834 A1, published November 26, 2025. Title: Method for production of cannabinoids in plants. Applicant: Quorum Biomedical S.L. The sequence listing filed with the application follows.

SEQUENCE LISTING (73 sequences)

SEQ ID NO: 1 - protein, 544 aa, Cannabis sp.
MKCSTFSFWFVCKIIFFFFSFNIQTSIANPRENFLKCFSQYIPNNATNLKLVYTQNNPLYMSVLNSTIHNLRFTSDTTPKPLVIVTPSHVSHIQGTILCSKKVGLQIRTRSGGHDSEGMSYISQVPFVIVDLRNMRSIKIDVHSQTAWVEAGATLGEVYYWVNEKNENLSLAAGYCPTVCAGGHFGGGGYGPLMRNYGLAADNIIDAHLVNVHGKVLDRKSMGEDLFWALRGGGAESFGIIVAWKIRLVAVPKSTMFSVKKIMEIHELVKLVNKWQNIAYKYDKDLLLMTHFITRNITDNQGKNKTAIHTYFSSVFLGGVDSLVDLMNKSFPELGIKKTDCRQLSWIDTIIFYSGVVNYDTDNFNKEILLDRSAGQNGAFKIKLDYVKKPIPESVFVQILEKLYEEDIGAGMYALYPYGGIMDEISESAIPFPHRAGILYELWYICSWEKQEDNEKHLNWIRNIYNFMTPYVSKNPRLAYLNYRDLDIGINDPKNPNNYTQARIWGEKYFGKNFDRLVKVKTLVDPNNFFRNEQSIPPLPRHRH

SEQ ID NO: 2 - protein, 545 aa, Cannabis sp.
MNCSAFSFWFVCKIIFFFLSFHIQISIANPRENFLKCFSKHIPNNVANPKLVYTQHDQLYMSILNSTIQNLRFISDTTPKPLVIVTPSNNSHIQATILCSKKVGLQIRTRSGGHDAEGMSYISQVPFVVVDLRNMHSIKIDVHSQTAWVEAGATLGEVYYWINEKNENLSFPGGYCPTVGVGGHFSGGGYGALMRNYGLAADNIIDAHLVNVDGKVLDRKSMGEDLFWAIRGGGGENFGIIAAWKIKLVDVPSKSTIFSVKKNMEIHGLVKLFNKWQNIAYKYDKDLVLMTHFITKNITDNHGKNKTTVHGYFSSIFHGGVDSLVDLMNKSFPELGIKKTDCKEFSWIDTTIFYSGVVNFNTANFKKEILLDRSAGKKTAFSIKLDYVKKPIPETAMVKILEKLYEEDVGAGMYVLYPYGGIMEEISESAIPFPHRAGIMYELWYTASWEKQEDNEKHINWVRSVYNFTTPYVSQNPRLAYLNYRDLDLGKTNHASPNNYTQARIWGEKYFGKNFNRLVKVKTKVDPNNFFRNEQSIPPLPPHHH

SEQ ID NO: 3 - DNA, 1635 bp, synthetic construct
  source 1..1635: mol_type = other DNA
atgaagtgctcaacattctccttttggtttgtttgcaagataatatttttctttttctcattcaatatccaaacttccattgctaatcctcgagaaaacttccttaaatgcttctcgcaatatattcccaataatgcaacaaatctaaaactcgtatacactcaaaacaacccattgtatatgtctgtcctaaattcgacaatacacaatcttagattcacctctgacacaaccccaaaaccacttgttatcgtcactccttcacatgtctctcatatccaaggcactattctatgctccaagaaagttggcttgcagattcgaactcgaagtggtggtcatgattctgagggcatgtcctacatatctcaagtcccatttgttatagtagacttgagaaacatgcgttcaatcaaaatagatgttcatagccaaactgcatgggttgaagccggagctacccttggagaagtttattattgggttaatgagaaaaatgagaatcttagtttggcggctgggtattgccctactgtttgcgcaggtggacactttggtggaggaggctatggaccattgatgagaaactatggcctcgcggctgataatatcattgatgcacacttagtcaacgttcatggaaaagtgctagatcgaaaatctatgggggaagatctcttttgggctttacgtggtggtggagcagaaagcttcggaatcattgtagcatggaaaattagactggttgctgtcccaaagtctactatgtttagtgttaaaaagatcatggagatacatgagcttgtcaagttagttaacaaatggcaaaatattgcttacaagtatgacaaagatttattactcatgactcacttcataactaggaacattacagataatcaagggaagaataagacagcaatacacacttacttctcttcagttttccttggtggagtggatagtctagtcgacttgatgaacaagagttttcctgagttgggtattaaaaaaacggattgcagacaattgagctggattgatactatcatcttctatagtggtgttgtaaattacgacactgataattttaacaaggaaattttgcttgatagatccgctgggcagaacggtgctttcaagattaagttagactacgttaagaaaccaattccagaatctgtatttgtccaaattttggaaaaattatatgaagaagatataggagctgggatgtatgcgttgtacccttacggtggtataatggatgagatttcagaatcagcaattccattccctcatcgagctggaatcttgtatgagttatggtacatatgtagttgggagaagcaagaagataacgaaaagcatctaaactggattagaaatatttataacttcatgactccttatgtgtccaaaaatccaagattggcatatctcaattatagagaccttgatataggaataaatgatcccaagaatccaaataattacacacaagcacgtatttggggtgagaagtattttggtaaaaattttgacaggctagtaaaagtgaaaaccctggttgatcccaataacttttttagaaacgaacaaagcatcccacctcttccacggcatcgtcattaa

SEQ ID NO: 4 - DNA, 306 bp, synthetic construct
  source 1..306: mol_type = other DNA
tgattcttatcacttcgtaaaaaaaagatagaaagatccataaataaatatttgctagtcctttctttccatagtcaacttcaatatggcatcttagcttctttccatcaacaaatgatgctcaactacttaatgtacaatttatatttatttttaataagggatgcacctaacaatacaatgatgcctaatttttgtgaattttttttaccacatgacttaatgatatcaaattatgaaatatttagttaatttatttgcccctgctccaatatataaagctataaataggatagttcttaatcc

SEQ ID NO: 5 - DNA, 23 bp, synthetic construct
  source 1..23: mol_type = other DNA
ctatttatagctttatatattgg

SEQ ID NO: 6 - DNA, 23 bp, synthetic construct
  source 1..23: mol_type = other DNA
atagctttatatattggagcagg

SEQ ID NO: 7 - DNA, 23 bp, synthetic construct
  source 1..23: mol_type = other DNA
tagctttatatattggagcaggg

SEQ ID NO: 8 - DNA, 23 bp, synthetic construct
  source 1..23: mol_type = other DNA
agctttatatattggagcagggg

SEQ ID NO: 9 - DNA, 23 bp, synthetic construct
  source 1..23: mol_type = other DNA
tttgatatcattaagtcatgtgg

SEQ ID NO: 10 - DNA, 23 bp, synthetic construct
  source 1..23: mol_type = other DNA
aaaaaaaattcacaaaaattagg

SEQ ID NO: 11 - DNA, 23 bp, synthetic construct
  source 1..23: mol_type = other DNA
ttaggcatcattgtattgttagg

SEQ ID NO: 12 - DNA, 23 bp, synthetic construct
  source 1..23: mol_type = other DNA
agttgagcatcatttgttgatgg

SEQ ID NO: 13 - DNA, 23 bp, synthetic construct
  source 1..23: mol_type = other DNA
tgccatattgaagttgactatgg

SEQ ID NO: 14 - DNA, 23 bp, synthetic construct
  source 1..23: mol_type = other DNA
gaagttgactatggaaagaaagg

SEQ ID NO: 15 - DNA, 23 bp, synthetic construct
  source 1..23: mol_type = other DNA
gactagcaaatatttatttatgg

SEQ ID NO: 16 - DNA, 23 bp, synthetic construct
  source 1..23: mol_type = other DNA
caatatataaagctataaatagg

SEQ ID NO: 17 - DNA, 23 bp, synthetic construct
  source 1..23: mol_type = other DNA
tttatatttatttttaataaggg

SEQ ID NO: 18 - DNA, 23 bp, synthetic construct
  source 1..23: mol_type = other DNA
atttatatttatttttaataagg

SEQ ID NO: 19 - DNA, 23 bp, synthetic construct
  source 1..23: mol_type = other DNA
ttccatagtcaacttcaatatgg

SEQ ID NO: 20 - protein, 1368 aa, synthetic construct
MDKKYSIGLAIGTNSVGWAVITDEYKVPSKKFKVLGNTDRHSIKKNLIGALLFDSGETAEATRLKRTARRRYTRRKNRICYLQEIFSNEMAKVDDSFFHRLEESFLVEEDKKHERHPIFGNIVDEVAYHEKYPTIYHLRKKLVDSTDKADLRLIYLALAHMIKFRGHFLIEGDLNPDNSDVDKLFIQLVQTYNQLFEENPINASGVDAKAILSARLSKSRRLENLIAQLPGEKKNGLFGNLIALSLGLTPNFKSNFDLAEDAKLQLSKDTYDDDLDNLLAQIGDQYADLFLAAKNLSDAILLSDILRVNTEITKAPLSASMIKRYDEHHQDLTLLKALVRQQLPEKYKEIFFDQSKNGYAGYIDGGASQEEFYKFIKPILEKMDGTEELLVKLNREDLLRKQRTFDNGSIPHQIHLGELHAILRRQEDFYPFLKDNREKIEKILTFRIPYYVGPLARGNSRFAWMTRKSEETITPWNFEEVVDKGASAQSFIERMTNFDKNLPNEKVLPKHSLLYEYFTVYNELTKVKYVTEGMRKPAFLSGEQKKAIVDLLFKTNRKVTVKQLKEDYFKKIECFDSVEISGVEDRFNASLGTYHDLLKIIKDKDFLDNEENEDILEDIVLTLTLFEDREMIEERLKTYAHLFDDKVMKQLKRRRYTGWGRLSRKLINGIRDKQSGKTILDFLKSDGFANRNFMQLIHDDSLTFKEDIQKAQVSGQGDSLHEHIANLAGSPAIKKGILQTVKVVDELVKVMGRHKPENIVIEMARENQTTQKGQKNSRERMKRIEEGIKELGSQILKEHPVENTQLQNEKLYLYYLQNGRDMYVDQELDINRLSDYDVDAIVPQSFLKDDSIDNKVLTRSDKNRGKSDNVPSEEVVKKMKNYWRQLLNAKLITQRKFDNLTKAERGGLSELDKAGFIKRQLVETRQITKHVAQILDSRMNTKYDENDKLIREVKVITLKSKLVSDFRKDFQFYKVREINNYHHAHDAYLNAVVGTALIKKYPKLESEFVYGDYKVYDVRKMIAKSEQEIGKATAKYFFYSNIMNFFKTEITLANGEIRKRPLIETNGETGEIVWDKGRDFATVRKVLSMPQVNIVKKTEVQTGGFSKESILPKRNSDKLIARKKDWDPKKYGGFDSPTVAYSVLVVAKVEKGKSKKLKSVKELLGITIMERSSFEKNPIDFLEAKGYKEVKKDLIIKLPKYSLFELENGRKRMLASAGELQKGNELALPSKYVNFLYLASHYEKLKGSPEDNEQKQLFVEQHKHYLDEIIEQISEFSKRVILADANLDKVLSAYNKHRDKPIREQAENIIHLFTLTNLGAPAAFKYFDTTIDRKRYTSTKEVLDATLIHQSITGLYETRIDLSQLGGD

SEQ ID NO: 21 - DNA, 346 bp, synthetic construct
  source 1..346: mol_type = other DNA
tgagacttttcaacaaagggtaatatccggaaacctcctcggattccattgcccagctatctgtcactttattgtgaagatagtggaaaaggaaggtggctcctacaaatgccatcattgcgataaaggaaaggccatcgttgaagatgcctctgccgacagtggtcccaaagatggacccccacccacgaggagcatcgtggaaaaagaagacgttccaaccacgtcttcaaagcaagtggattgatgtgatatctccactgacgtaagggatgacgcacaatcccactatccttcgcaagacccttcctctatataaggaagttcatttcatttggagagaaca

SEQ ID NO: 22 - DNA, 253 bp, synthetic construct
  source 1..253: mol_type = other DNA
gatcgttcaaacatttggcaataaagtttcttaagattgaatcctgttgccggtcttgcgatgattatcatataatttctgttgaattacgttaagcatgtaataattaacatgtaatgcatgacgttatttatgagatgggtttttatgattagagtcccgcaattatacatttaatacgcgatagaaaacaaaatatagcgcgcaaactaggataaattatcgcgcgcggtgtcatctatgttactagatc

SEQ ID NO: 23 - DNA, 18 bp, synthetic construct
  source 1..18: mol_type = other DNA
catcaccatcaccatcac

SEQ ID NO: 24 - DNA, 630 bp, synthetic construct
  source 1..630: mol_type = other DNA
atgaaggttatcgctgtacttaaccagaaaggcgggtcaggcaagacgaccatcgcaacccatctagcccgcgccctgcaactcgccggggccgatgttctgttagtcgattccgatccccagggcagtgcccgcgattgggcggccgtgcgggaagatcaaccgctaaccgttgtcggcatcgaccgcccgacgattgaccgcgacgtgaaggccatcggccggcgcgacttcgtagtgatcgacggagcgccccaggcggcggacttggctgtgtccgcgatcaaggcagccgacttcgtgctgattccggtgcagccaagcccttacgacatatgggccaccgccgacctggtggagctggttaagcagcgcattgaggtcacggatggaaggctacaagcggcctttgtcgtgtcgcgggcgatcaaaggcacgcgcatcggcggtgaggttgccgaggcgctggccgggtacgagctgcccattcttgagtcccgtatcacgcagcgcgtgagctacccaggcactgccgccgccggcacaaccgttcttgaatcagaacccgagggcgacgctgcccgcgaggtccaggcgctggccgctgaaattaaatcaaaactcatttga

SEQ ID NO: 25 - DNA, 1074 bp, synthetic construct
  source 1..1074: mol_type = other DNA
gtgagcggtcgcaaaccatccggcccggtacaaatcggcgcggcgctgggtgatgacctggtggagaagttgaaggccgcgcaggccgcccagcggcaacgcatcgaggcagaagcacgccccggtgaatcgtggcaagcggccgctgatcgaatccgcaaagaatcccggcaaccgccggcagccggtgcgccgtcgattaggaagccgcccaagggcgacgagcaaccagattttttcgttccgatgctctatgacgtgggcacccgcgatagtcgcagcatcatggacgtggccgttttccgtctgtcgaagcgtgaccgacgagctggcgaggtgatccgctacgagcttccagacgggcacgtagaggtttccgcagggccggccggcatggccagtgtgtgggattacgacctggtactgatggcggtttcccatctaaccgaatccatgaaccgataccgggaagggaagggagacaagcccggccgcgtgttccgtccacacgttgcggacgtactcaagttctgccggcgagccgatggcggaaagcagaaagacgacctggtagaaacctgcattcggttaaacaccacgcacgttgccatgcagcgtacgaagaaggccaagaacggccgcctggtgacggtatccgagggtgaagccttgattagccgctacaagatcgtaaagagcgaaaccgggcggccggagtacatcgagatcgagctagctgattggatgtaccgcgagatcacagaaggcaagaacccggacgtgctgacggttcaccccgattactttttgatcgatcccggcatcggccgttttctctaccgcctggcacgccgcgccgcaggcaaggcagaagccagatggttgttcaagacgatctacgaacgcagtggcagcgccggagagttcaagaagttctgtttcaccgtgcgcaagctgatcgggtcaaatgacctgccggagtacgatttgaaggaggaggcggggcaggctggcccgatcctagtcatgcgctaccgcaacctgatcgagggcgaagcatccgccggttcctaa

SEQ ID NO: 26 - DNA, 141 bp, synthetic construct
  source 1..141: mol_type = other DNA
cgcagccatgacccagtcacgtagcgatagcggagtgtatactggcttaactatgcggcatcagagcagattgtactgagagtgcaccatatgcggtgtgaaataccgcacagatgcgtaaggagaaaataccgcatcagg

SEQ ID NO: 27 - DNA, 195 bp, synthetic construct
  source 1..195: mol_type = other DNA
tgtggatagcacgtacattgggaacccaaagccgtacattgggaaccggaacccgtacattgggaacccaaagccgtacattgggaaccggtcacacatgtaagtgactgatataaaagagaaaaaaggcgatttttccgcctaaaactctttaaaacttattaaaactcttaaaacccgcctggcctgtgcata

SEQ ID NO: 28 - DNA, 589 bp, synthetic construct
  source 1..589: mol_type = other DNA
tttccataggctccgcccccctgacgagcatcacaaaaatcgacgctcaagtcagaggtggcgaaacccgacaggactataaagataccaggcgtttccccctggaagctccctcgtgcgctctcctgttccgaccctgccgcttaccggatacctgtccgcctttctcccttcgggaagcgtggcgctttctcatagctcacgctgtaggtatctcagttcggtgtaggtcgttcgctccaagctgggctgtgtgcacgaaccccccgttcagcccgaccgctgcgccttatccggtaactatcgtcttgagtccaacccggtaagacacgacttatcgccactggcagcagccactggtaacaggattagcagagcgaggtatgtaggcggtgctacagagttcttgaagtggtggcctaactacggctacactagaaggacagtatttggtatctgcgctctgctgaagccagttaccttcggaaaaagagttggtagctcttgatccggcaaacaaaccaccgctggtagcggtggtttttttgtttgcaagcagcagattacgcgcagaaaaaaaggatctcaa

SEQ ID NO: 29 - DNA, 795 bp, synthetic construct
  source 1..795: mol_type = other DNA
ctaaaacaattcatccagtaaaatataatattttattttctcccaatcaggcttgatccccagtaagtcaaaaaatagctcgacatactgttcttccccgatatcctccctgatcgaccggacgcagaaggcaatgtcataccacttgtccgccctgccgcttctcccaagatcaataaagccacttactttgccatctttcacaaagatgttgctgtctcccaggtcgccgtgggaaaagacaagttcctcttcgggcttttccgtctttaaaaaatcatacagctcgcgcggatctttaaatggagtgtcttcttcccagttttcgcaatccacatcggccagatcgttattcagtaagtaatccaattcggctaagcggctgtctaagctattcgtatagggacaatccgatatgtcgatggagtgaaagagcctgatgcactccgcatacagctcgataatcttttcagggctttgttcatcttcatactcttccgagcaaaggacgccatcggcctcactcatgagcagattgctccagccatcatgccgttcaaagtgcaggacctttggaacaggcagctttccttccagccatagcatcatgtccttttcccgttccacatcataggtggtccctttataccggctgtccgtcatttttaaatataggttttcattttctcccaccagcttatataccttagcaggagacattccttccgtatcttttacgcagcggtatttttcgatcagttttttcaattccggtgatattctcattttagccat

SEQ ID NO: 30 - DNA, 9737 bp, synthetic construct
  source 1..9737: mol_type = other DNA
catggctactactaagcatttggctcttgccatccttgtcctccttagcattggtatgaccaccagtgcaagaaccctcctagatctgagggtaaatttctagtttttctccttcattttcttggttaggacccttttctctttttatttttttgagctttgatctttctttaaactgatctattttttaattgattggttatggtgtaaatattacatagctttaactgataatctgattactttatttcgtgtgtctatgatgatgatgatagttacagaaccgacgaactagtctgtacccgatcaacaccgagacccgtggcgtcttcgacctcaatggcgtctggaacttcaagctggactacgggaaaggactggaagagaagtggtacgaaagcaagctgaccgacactattagtatggccgtcccaagcagttacaatgacattggcgtgaccaaggaaatccgcaaccatatcggatatgtctggtacgaacgtgagttcacggtgccggcctatctgaaggatcagcgtatcgtgctccgcttcggctctgcaactcacaaagcaattgtctatgtcaatggtgagctggtcgtggagcacaagggcggattcctgccattcgaagcggaaatcaacaactcgctgcgtgatggcatgaatcgcgtcaccgtcgccgtggacaacatcctcgacgatagcaccctcccggtggggctgtacagcgagcgccacgaagagggcctcggaaaagtcattcgtaacaagccgaacttcgacttcttcaactatgcaggcctgcaccgtccggtgaaaatctacacgaccccgtttacgtacgtcgaggacatctcggttgtgaccgacttcaatggcccaaccgggactgtgacctatacggtggactttcaaggcaaagccgagaccgtgaaagtgtcggtcgtggatgaggaaggcaaagtggtcgcaagcaccgagggcctgagcggtaacgtggagattccgaatgtcatcctctgggaaccactgaacacgtatctctaccagatcaaagtggaactggtgaacgacggactgaccatcgatgtctatgaagagccgttcggcgtgcggaccgtggaagtcaacgacggcaagttcctcatcaacaacaaaccgttctacttcaagggctttggcaaacatgaggacactcctatcaacggccgtggctttaacgaagcgagcaatgtgatggatttcaatatcctcaaatggatcggcgccaacagcttccggaccgcacactatccgtactctgaagagttgatgcgtcttgcggatcgcgagggtctggtcgtgatcgacgagactccggcagttggcgtgcacctcaacttcatggccaccacgggactcggcgaaggcagcgagcgcgtcagtacctgggagaagattcggacgtttgagcaccatcaagacgttctccgtgaactggtgtctcgtgacaagaaccatccaagcgtcgtgatgtggagcatcgccaacgaggcggcgactgaggaagagggcgcgtacgagtacttcaagccgttggtggagctgaccaaggaactcgacccacagaagcgtccggtcacgatcgtgctgtttgtgatggctaccccggagacggacaaagtcgccgaactgattgacgtcatcgcgctcaatcgctataacggatggtacttcgatggcggtgatctcgaagcggccaaagtccatctccgccaggaatttcacgcgtggaacaagcgttgcccaggaaagccgatcatgatcactgagtacggcgcagacaccgttgcgggctttcacgacattgatccagtgatgttcaccgaggaatatcaagtcgagtactaccaggcgaaccacgtcgtgttcgatgagtttgagaacttcgtgggtgagcaagcgtggaacttcgcggacttcgcgacctctcagggcgtgatgcgcgtccaaggaaacaagaagggcgtgttcactcgtgaccgcaagccgaagctcgccgcgcacgtctttcgcgagcgctggaccaacattccagatttcggctacaagaacgctagccatcaccatcaccatcacgtgtgaattggtgaccagctcgaatttccccgatcgttcaaacatttggcaataaagtttcttaagattgaatcctgttgccggtcttgcgatgattatcatataatttctgttgaattacgttaagcatgtaataattaacatgtaatgcatgacgttatttatgagatgggtttttatgattagagtcccgcaattatacatttaatacgcgatagaaaacaaaatatagcgcgcaaactaggataaattatcgcgcgcggtgtcatctatgttactagatcgggaattaaactatcagtgtttgacaggatatattggcgggtaaacctaagagaaaagagcgtttattagaataacggatatttaaaagggcgtgaaaaggtttatccgttcgtccatttgtatgtgcatgccaaccacagggttcccctcgggatcaaagtactttgatccaacccctccgctgctatagtgcagtcggcttctgacgttcagtgcagccgtcttctgaaaacgacatgtcgcacaagtcctaagttacgcgacaggctgccgccctgcccttttcctggcgttttcttgtcgcgtgttttagtcgcataaagtagaatacttgcgactagaaccggagacattacgccatgaacaagagcgccgccgctggcctgctgggctatgcccgcgtcagcaccgacgaccaggacttgaccaaccaacgggccgaactgcacgcggccggctgcaccaagctgttttccgagaagatcaccggcaccaggcgcgaccgcccggagctggccaggatgcttgaccacctacgccctggcgacgttgtgacagtgaccaggctagaccgcctggcccgcagcacccgcgacctactggacattgccgagcgcatccaggaggccggcgcgggcctgcgtagcctggcagagccgtgggccgacaccaccacgccggccggccgcatggtgttgaccgtgttcgccggcattgccgagttcgagcgttccctaatcatcgaccgcacccggagcgggcgcgaggccgccaaggcccgaggcgtgaagtttggcccccgccctaccctcaccccggcacagatcgcgcacgcccgcgagctgatcgaccaggaaggccgcaccgtgaaagaggcggctgcactgcttggcgtgcatcgctcgaccctgtaccgcgcacttgagcgcagcgaggaagtgacgcccaccgaggccaggcggcgcggtgccttccgtgaggacgcattgaccgaggccgacgccctggcggccgccgagaatgaacgccaagaggaacaagcatgaaaccgcaccaggacggccaggacgaaccgtttttcattaccgaagagatcgaggcggagatgatcgcggccgggtacgtgttcgagccgcccgcgcacgtctcaaccgtgcggctgcatgaaatcctggccggtttgtctgatgccaagctggcggcctggccggccagcttggccgctgaagaaaccgagcgccgccgtctaaaaaggtgatgtgtatttgagtaaaacagcttgcgtcatgcggtcgctgcgtatatgatgcgatgagtaaataaacaaatacgcaaggggaacgcatgaaggttatcgctgtacttaaccagaaaggcgggtcaggcaagacgaccatcgcaacccatctagcccgcgccctgcaactcgccggggccgatgttctgttagtcgattccgatccccagggcagtgcccgcgattgggcggccgtgcgggaagatcaaccgctaaccgttgtcggcatcgaccgcccgacgattgaccgcgacgtgaaggccatcggccggcgcgacttcgtagtgatcgacggagcgccccaggcggcggacttggctgtgtccgcgatcaaggcagccgacttcgtgctgattccggtgcagccaagcccttacgacatatgggccaccgccgacctggtggagctggttaagcagcgcattgaggtcacggatggaaggctacaagcggcctttgtcgtgtcgcgggcgatcaaaggcacgcgcatcggcggtgaggttgccgaggcgctggccgggtacgagctgcccattcttgagtcccgtatcacgcagcgcgtgagctacccaggcactgccgccgccggcacaaccgttcttgaatcagaacccgagggcgacgctgcccgcgaggtccaggcgctggccgctgaaattaaatcaaaactcatttgagttaatgaggtaaagagaaaatgagcaaaagcacaaacacgctaagtgccggccgtccgagcgcacgcagcagcaaggctgcaacgttggccagcctggcagacacgccagccatgaagcgggtcaactttcagttgccggcggaggatcacaccaagctgaagatgtacgcggtacgccaaggcaagaccattaccgagctgctatctgaatacatcgcgcagctaccagagtaaatgagcaaatgaataaatgagtagatgaattttagcggctaaaggaggcggcatggaaaatcaagaacaaccaggcaccgacgccgtggaatgccccatgtgtggaggaacgggcggttggccaggcgtaagcggctgggttgtctgccggccctgcaatggcactggaacccccaagcccgaggaatcggcgtgagcggtcgcaaaccatccggcccggtacaaatcggcgcggcgctgggtgatgacctggtggagaagttgaaggccgcgcaggccgcccagcggcaacgcatcgaggcagaagcacgccccggtgaatcgtggcaagcggccgctgatcgaatccgcaaagaatcccggcaaccgccggcagccggtgcgccgtcgattaggaagccgcccaagggcgacgagcaaccagattttttcgttccgatgctctatgacgtgggcacccgcgatagtcgcagcatcatggacgtggccgttttccgtctgtcgaagcgtgaccgacgagctggcgaggtgatccgctacgagcttccagacgggcacgtagaggtttccgcagggccggccggcatggccagtgtgtgggattacgacctggtactgatggcggtttcccatctaaccgaatccatgaaccgataccgggaagggaagggagacaagcccggccgcgtgttccgtccacacgttgcggacgtactcaagttctgccggcgagccgatggcggaaagcagaaagacgacctggtagaaacctgcattcggttaaacaccacgcacgttgccatgcagcgtacgaagaaggccaagaacggccgcctggtgacggtatccgagggtgaagccttgattagccgctacaagatcgtaaagagcgaaaccgggcggccggagtacatcgagatcgagctagctgattggatgtaccgcgagatcacagaaggcaagaacccggacgtgctgacggttcaccccgattactttttgatcgatcccggcatcggccgttttctctaccgcctggcacgccgcgccgcaggcaaggcagaagccagatggttgttcaagacgatctacgaacgcagtggcagcgccggagagttcaagaagttctgtttcaccgtgcgcaagctgatcgggtcaaatgacctgccggagtacgatttgaaggaggaggcggggcaggctggcccgatcctagtcatgcgctaccgcaacctgatcgagggcgaagcatccgccggttcctaatgtacggagcagatgctagggcaaattgccctagcaggggaaaaaggtcgaaaaggtctctttcctgtggatagcacgtacattgggaacccaaagccgtacattgggaaccggaacccgtacattgggaacccaaagccgtacattgggaaccggtcacacatgtaagtgactgatataaaagagaaaaaaggcgatttttccgcctaaaactctttaaaacttattaaaactcttaaaacccgcctggcctgtgcataactgtctggccagcgcacagccgaagagctgcaaaaagcgcctacccttcggtcgctgcgctccctacgccccgccgcttcgcgtcggcctatcgcggccgctggccgctcaaaaatggctggcctacggccaggcaatctaccagggcgcggacaagccgcgccgtcgccactcgaccgccggcgcccacatcaaggcaccctgcctcgcgcgtttcggtgatgacggtgaaaacctctgacacatgcagctcccggagacggtcacagcttgtctgtaagcggatgccgggagcagacaagcccgtcagggcgcgtcagcgggtgttggcgggtgtcggggcgcagccatgacccagtcacgtagcgatagcggagtgtatactggcttaactatgcggcatcagagcagattgtactgagagtgcaccatatgcggtgtgaaataccgcacagatgcgtaaggagaaaataccgcatcaggcgctcttccgcttcctcgctcactgactcgctgcgctcggtcgttcggctgcggcgagcggtatcagctcactcaaaggcggtaatacggttatccacagaatcaggggataacgcaggaaagaacatgtgagcaaaaggccagcaaaaggccaggaaccgtaaaaaggccgcgttgctggcgtttttccataggctccgcccccctgacgagcatcacaaaaatcgacgctcaagtcagaggtggcgaaacccgacaggactataaagataccaggcgtttccccctggaagctccctcgtgcgctctcctgttccgaccctgccgcttaccggatacctgtccgcctttctcccttcgggaagcgtggcgctttctcatagctcacgctgtaggtatctcagttcggtgtaggtcgttcgctccaagctgggctgtgtgcacgaaccccccgttcagcccgaccgctgcgccttatccggtaactatcgtcttgagtccaacccggtaagacacgacttatcgccactggcagcagccactggtaacaggattagcagagcgaggtatgtaggcggtgctacagagttcttgaagtggtggcctaactacggctacactagaaggacagtatttggtatctgcgctctgctgaagccagttaccttcggaaaaagagttggtagctcttgatccggcaaacaaaccaccgctggtagcggtggtttttttgtttgcaagcagcagattacgcgcagaaaaaaaggatctcaagaagatcctttgatcttttctacggggtctgacgctcagtggaacgaaaactcacgttaagggattttggtcatgcattctaggtactaaaacaattcatccagtaaaatataatattttattttctcccaatcaggcttgatccccagtaagtcaaaaaatagctcgacatactgttcttccccgatatcctccctgatcgaccggacgcagaaggcaatgtcataccacttgtccgccctgccgcttctcccaagatcaataaagccacttactttgccatctttcacaaagatgttgctgtctcccaggtcgccgtgggaaaagacaagttcctcttcgggcttttccgtctttaaaaaatcatacagctcgcgcggatctttaaatggagtgtcttcttcccagttttcgcaatccacatcggccagatcgttattcagtaagtaatccaattcggctaagcggctgtctaagctattcgtatagggacaatccgatatgtcgatggagtgaaagagcctgatgcactccgcatacagctcgataatcttttcagggctttgttcatcttcatactcttccgagcaaaggacgccatcggcctcactcatgagcagattgctccagccatcatgccgttcaaagtgcaggacctttggaacaggcagctttccttccagccatagcatcatgtccttttcccgttccacatcataggtggtccctttataccggctgtccgtcatttttaaatataggttttcattttctcccaccagcttatataccttagcaggagacattccttccgtatcttttacgcagcggtatttttcgatcagttttttcaattccggtgatattctcattttagccatttattatttccttcctcttttctacagtatttaaagataccccaagaagctaattataacaagacgaactccaattcactgttccttgcattctaaaaccttaaataccagaaaacagctttttcaaagttgttttcaaagttggcgtataacatagtatcgacggagccgattttgaaaccgcggtgatcacaggcagcaacgctctgtcatcgttacaatcaacatgctaccctccgcgagatcatccgtgtttcaaacccggcagcttagttgccgttcttccgaatagcatcggtaacatgagcaaagtctgccgccttacaacggctctcccgctgacgccgtcccggactgatgggctgcctgtatcgagtggtgattttgtgccgagctgccggtcggggagctgttggctggctggtggcaggatatattgtggtgtaaacaaattgacgcttagacaacttaataacacattgcggacgtttttaatgtactgaattaacgccgaattaatgtgagttagctcactcattaggcaccccaggctttacactttatgcttccggctcgtatgttgtgtggaattgtgagcggataacaatttcacacaggaaacagctatgaccatgattacgaattcgagctcggtacccggggatcctctagagtcgacctgcaggcatgcaagcttggcactggccgtcgttttacaacgtcgtgactgggaaaaccctggcgttacccaacttaatcgccttgcagcacatccccctttcgccagctggcgtaatagcgaagaggcccgcaccgatcgcccttcccaacagttgcgcagcctgaatggcgaatgctagagcagcttgagcttggatcagattgtcgtttcccgccttcagtttagcttcatggagtcaaagattcaaatagaggacctaacagaactcgccgtaaagactggcgaacagttcatacagagtctcttacgactcaatgacaagaagaaaatcttcgtcaacatggtggagcacgacacacttgtctactccaaaaatatcaaagatacagtctcagaagaccaaagggcaattgagacttttcaacaaagggtaatatccggaaacctcctcggattccattgcccagctatctgtcactttattgtgaagatagtggaaaaggaaggtggctcctacaaatgccatcattgcgataaaggaaaggccatcgttgaagatgcctctgccgacagtggtcccaaagatggacccccacccacgaggagcatcgtggaaaaagaagacgttccaaccacgtcttcaaagcaagtggattgatgtgatatctccactgacgtaagggatgacgcacaatcccactatccttcgcaagacccttcctctatataaggaagttcatttcatttggagagaacacgggggactcttgac

SEQ ID NO: 31 - DNA, 9279 bp, synthetic construct
  source 1..9279: mol_type = other DNA
catgaagtgctcaacattctccttttggtttgtttgcaagataatatttttctttttctcattcaatatccaaacttccattgctaatcctcgagaaaacttccttaaatgcttctcgcaatatattcccaataatgcaacaaatctaaaactcgtatacactcaaaacaacccattgtatatgtctgtcctaaattcgacaatacacaatcttagattcacctctgacacaaccccaaaaccacttgttatcgtcactccttcacatgtctctcatatccaaggcactattctatgctccaagaaagttggcttgcagattcgaactcgaagtggtggtcatgattctgagggcatgtcctacatatctcaagtcccatttgttatagtagacttgagaaacatgcgttcaatcaaaatagatgttcatagccaaactgcatgggttgaagccggagctacccttggagaagtttattattgggttaatgagaaaaatgagaatcttagtttggcggctgggtattgccctactgtttgcgcaggtggacactttggtggaggaggctatggaccattgatgagaaactatggcctcgcggctgataatatcattgatgcacacttagtcaacgttcatggaaaagtgctagatcgaaaatctatgggggaagatctcttttgggctttacgtggtggtggagcagaaagcttcggaatcattgtagcatggaaaattagactggttgctgtcccaaagtctactatgtttagtgttaaaaagatcatggagatacatgagcttgtcaagttagttaacaaatggcaaaatattgcttacaagtatgacaaagatttattactcatgactcacttcataactaggaacattacagataatcaagggaagaataagacagcaatacacacttacttctcttcagttttccttggtggagtggatagtctagtcgacttgatgaacaagagttttcctgagttgggtattaaaaaaacggattgcagacaattgagctggattgatactatcatcttctatagtggtgttgtaaattacgacactgataattttaacaaggaaattttgcttgatagatccgctgggcagaacggtgctttcaagattaagttagactacgttaagaaaccaattccagaatctgtatttgtccaaattttggaaaaattatatgaagaagatataggagctgggatgtatgcgttgtacccttacggtggtataatggatgagatttcagaatcagcaattccattccctcatcgagctggaatcttgtatgagttatggtacatatgtagttgggagaagcaagaagataacgaaaagcatctaaactggattagaaatatttataacttcatgactccttatgtgtccaaaaatccaagattggcatatctcaattatagagaccttgatataggaataaatgatcccaagaatccaaataattacacacaagcacgtatttggggtgagaagtattttggtaaaaattttgacaggctagtaaaagtgaaaaccctggttgatcccaataacttttttagaaacgaacaaagcatcccacctcttccacggcatcgtcatgctagccatcaccatcaccatcacgtgtgaagcgatcgcttggtgaccagctcgaatttccccgatcgttcaaacatttggcaataaagtttcttaagattgaatcctgttgccggtcttgcgatgattatcatataatttctgttgaattacgttaagcatgtaataattaacatgtaatgcatgacgttatttatgagatgggtttttatgattagagtcccgcaattatacatttaatacgcgatagaaaacaaaatatagcgcgcaaactaggataaattatcgcgcgcggtgtcatctatgttactagatcgggaattaaactatcagtgtttgacaggatatattggcgggtaaacctaagagaaaagagcgtttattagaataacggatatttaaaagggcgtgaaaaggtttatccgttcgtccatttgtatgtgcatgccaaccacagggttcccctcgggatcaaagtactttgatccaacccctccgctgctatagtgcagtcggcttctgacgttcagtgcagccgtcttctgaaaacgacatgtcgcacaagtcctaagttacgcgacaggctgccgccctgcccttttcctggcgttttcttgtcgcgtgttttagtcgcataaagtagaatacttgcgactagaaccggagacattacgccatgaacaagagcgccgccgctggcctgctgggctatgcccgcgtcagcaccgacgaccaggacttgaccaaccaacgggccgaactgcacgcggccggctgcaccaagctgttttccgagaagatcaccggcaccaggcgcgaccgcccggagctggccaggatgcttgaccacctacgccctggcgacgttgtgacagtgaccaggctagaccgcctggcccgcagcacccgcgacctactggacattgccgagcgcatccaggaggccggcgcgggcctgcgtagcctggcagagccgtgggccgacaccaccacgccggccggccgcatggtgttgaccgtgttcgccggcattgccgagttcgagcgttccctaatcatcgaccgcacccggagcgggcgcgaggccgccaaggcccgaggcgtgaagtttggcccccgccctaccctcaccccggcacagatcgcgcacgcccgcgagctgatcgaccaggaaggccgcaccgtgaaagaggcggctgcactgcttggcgtgcatcgctcgaccctgtaccgcgcacttgagcgcagcgaggaagtgacgcccaccgaggccaggcggcgcggtgccttccgtgaggacgcattgaccgaggccgacgccctggcggccgccgagaatgaacgccaagaggaacaagcatgaaaccgcaccaggacggccaggacgaaccgtttttcattaccgaagagatcgaggcggagatgatcgcggccgggtacgtgttcgagccgcccgcgcacgtctcaaccgtgcggctgcatgaaatcctggccggtttgtctgatgccaagctggcggcctggccggccagcttggccgctgaagaaaccgagcgccgccgtctaaaaaggtgatgtgtatttgagtaaaacagcttgcgtcatgcggtcgctgcgtatatgatgcgatgagtaaataaacaaatacgcaaggggaacgcatgaaggttatcgctgtacttaaccagaaaggcgggtcaggcaagacgaccatcgcaacccatctagcccgcgccctgcaactcgccggggccgatgttctgttagtcgattccgatccccagggcagtgcccgcgattgggcggccgtgcgggaagatcaaccgctaaccgttgtcggcatcgaccgcccgacgattgaccgcgacgtgaaggccatcggccggcgcgacttcgtagtgatcgacggagcgccccaggcggcggacttggctgtgtccgcgatcaaggcagccgacttcgtgctgattccggtgcagccaagcccttacgacatatgggccaccgccgacctggtggagctggttaagcagcgcattgaggtcacggatggaaggctacaagcggcctttgtcgtgtcgcgggcgatcaaaggcacgcgcatcggcggtgaggttgccgaggcgctggccgggtacgagctgcccattcttgagtcccgtatcacgcagcgcgtgagctacccaggcactgccgccgccggcacaaccgttcttgaatcagaacccgagggcgacgctgcccgcgaggtccaggcgctggccgctgaaattaaatcaaaactcatttgagttaatgaggtaaagagaaaatgagcaaaagcacaaacacgctaagtgccggccgtccgagcgcacgcagcagcaaggctgcaacgttggccagcctggcagacacgccagccatgaagcgggtcaactttcagttgccggcggaggatcacaccaagctgaagatgtacgcggtacgccaaggcaagaccattaccgagctgctatctgaatacatcgcgcagctaccagagtaaatgagcaaatgaataaatgagtagatgaattttagcggctaaaggaggcggcatggaaaatcaagaacaaccaggcaccgacgccgtggaatgccccatgtgtggaggaacgggcggttggccaggcgtaagcggctgggttgtctgccggccctgcaatggcactggaacccccaagcccgaggaatcggcgtgagcggtcgcaaaccatccggcccggtacaaatcggcgcggcgctgggtgatgacctggtggagaagttgaaggccgcgcaggccgcccagcggcaacgcatcgaggcagaagcacgccccggtgaatcgtggcaagcggccgctgatcgaatccgcaaagaatcccggcaaccgccggcagccggtgcgccgtcgattaggaagccgcccaagggcgacgagcaaccagattttttcgttccgatgctctatgacgtgggcacccgcgatagtcgcagcatcatggacgtggccgttttccgtctgtcgaagcgtgaccgacgagctggcgaggtgatccgctacgagcttccagacgggcacgtagaggtttccgcagggccggccggcatggccagtgtgtgggattacgacctggtactgatggcggtttcccatctaaccgaatccatgaaccgataccgggaagggaagggagacaagcccggccgcgtgttccgtccacacgttgcggacgtactcaagttctgccggcgagccgatggcggaaagcagaaagacgacctggtagaaacctgcattcggttaaacaccacgcacgttgccatgcagcgtacgaagaaggccaagaacggccgcctggtgacggtatccgagggtgaagccttgattagccgctacaagatcgtaaagagcgaaaccgggcggccggagtacatcgagatcgagctagctgattggatgtaccgcgagatcacagaaggcaagaacccggacgtgctgacggttcaccccgattactttttgatcgatcccggcatcggccgttttctctaccgcctggcacgccgcgccgcaggcaaggcagaagccagatggttgttcaagacgatctacgaacgcagtggcagcgccggagagttcaagaagttctgtttcaccgtgcgcaagctgatcgggtcaaatgacctgccggagtacgatttgaaggaggaggcggggcaggctggcccgatcctagtcatgcgctaccgcaacctgatcgagggcgaagcatccgccggttcctaatgtacggagcagatgctagggcaaattgccctagcaggggaaaaaggtcgaaaaggtctctttcctgtggatagcacgtacattgggaacccaaagccgtacattgggaaccggaacccgtacattgggaacccaaagccgtacattgggaaccggtcacacatgtaagtgactgatataaaagagaaaaaaggcgatttttccgcctaaaactctttaaaacttattaaaactcttaaaacccgcctggcctgtgcataactgtctggccagcgcacagccgaagagctgcaaaaagcgcctacccttcggtcgctgcgctccctacgccccgccgcttcgcgtcggcctatcgcggccgctggccgctcaaaaatggctggcctacggccaggcaatctaccagggcgcggacaagccgcgccgtcgccactcgaccgccggcgcccacatcaaggcaccctgcctcgcgcgtttcggtgatgacggtgaaaacctctgacacatgcagctcccggagacggtcacagcttgtctgtaagcggatgccgggagcagacaagcccgtcagggcgcgtcagcgggtgttggcgggtgtcggggcgcagccatgacccagtcacgtagcgatagcggagtgtatactggcttaactatgcggcatcagagcagattgtactgagagtgcaccatatgcggtgtgaaataccgcacagatgcgtaaggagaaaataccgcatcaggcgctcttccgcttcctcgctcactgactcgctgcgctcggtcgttcggctgcggcgagcggtatcagctcactcaaaggcggtaatacggttatccacagaatcaggggataacgcaggaaagaacatgtgagcaaaaggccagcaaaaggccaggaaccgtaaaaaggccgcgttgctggcgtttttccataggctccgcccccctgacgagcatcacaaaaatcgacgctcaagtcagaggtggcgaaacccgacaggactataaagataccaggcgtttccccctggaagctccctcgtgcgctctcctgttccgaccctgccgcttaccggatacctgtccgcctttctcccttcgggaagcgtggcgctttctcatagctcacgctgtaggtatctcagttcggtgtaggtcgttcgctccaagctgggctgtgtgcacgaaccccccgttcagcccgaccgctgcgccttatccggtaactatcgtcttgagtccaacccggtaagacacgacttatcgccactggcagcagccactggtaacaggattagcagagcgaggtatgtaggcggtgctacagagttcttgaagtggtggcctaactacggctacactagaaggacagtatttggtatctgcgctctgctgaagccagttaccttcggaaaaagagttggtagctcttgatccggcaaacaaaccaccgctggtagcggtggtttttttgtttgcaagcagcagattacgcgcagaaaaaaaggatctcaagaagatcctttgatcttttctacggggtctgacgctcagtggaacgaaaactcacgttaagggattttggtcatgcattctaggtactaaaacaattcatccagtaaaatataatattttattttctcccaatcaggcttgatccccagtaagtcaaaaaatagctcgacatactgttcttccccgatatcctccctgatcgaccggacgcagaaggcaatgtcataccacttgtccgccctgccgcttctcccaagatcaataaagccacttactttgccatctttcacaaagatgttgctgtctcccaggtcgccgtgggaaaagacaagttcctcttcgggcttttccgtctttaaaaaatcatacagctcgcgcggatctttaaatggagtgtcttcttcccagttttcgcaatccacatcggccagatcgttattcagtaagtaatccaattcggctaagcggctgtctaagctattcgtatagggacaatccgatatgtcgatggagtgaaagagcctgatgcactccgcatacagctcgataatcttttcagggctttgttcatcttcatactcttccgagcaaaggacgccatcggcctcactcatgagcagattgctccagccatcatgccgttcaaagtgcaggacctttggaacaggcagctttccttccagccatagcatcatgtccttttcccgttccacatcataggtggtccctttataccggctgtccgtcatttttaaatataggttttcattttctcccaccagcttatataccttagcaggagacattccttccgtatcttttacgcagcggtatttttcgatcagttttttcaattccggtgatattctcattttagccatttattatttccttcctcttttctacagtatttaaagataccccaagaagctaattataacaagacgaactccaattcactgttccttgcattctaaaaccttaaataccagaaaacagctttttcaaagttgttttcaaagttggcgtataacatagtatcgacggagccgattttgaaaccgcggtgatcacaggcagcaacgctctgtcatcgttacaatcaacatgctaccctccgcgagatcatccgtgtttcaaacccggcagcttagttgccgttcttccgaatagcatcggtaacatgagcaaagtctgccgccttacaacggctctcccgctgacgccgtcccggactgatgggctgcctgtatcgagtggtgattttgtgccgagctgccggtcggggagctgttggctggctggtggcaggatatattgtggtgtaaacaaattgacgcttagacaacttaataacacattgcggacgtttttaatgtactgaattaacgccgaattaatgtgagttagctcactcattaggcaccccaggctttacactttatgcttccggctcgtatgttgtgtggaattgtgagcggataacaatttcacacaggaaacagctatgaccatgattacgaattcgagctcggtacccggggatcctctagagtcgacctgcaggcatgcaagcttggcactggccgtcgttttacaacgtcgtgactgggaaaaccctggcgttacccaacttaatcgccttgcagcacatccccctttcgccagctggcgtaatagcgaagaggcccgcaccgatcgcccttcccaacagttgcgcagcctgaatggcgaatgctagagcagcttgagcttggatcagattgtcgtttcccgccttcagtttagcttcatggagtcaaagattcaaatagaggacctaacagaactcgccgtaaagactggcgaacagttcatacagagtctcttacgactcaatgacaagaagaaaatcttcgtcaacatggtggagcacgacacacttgtctactccaaaaatatcaaagatacagtctcagaagaccaaagggcaattgagacttttcaacaaagggtaatatccggaaacctcctcggattccattgcccagctatctgtcactttattgtgaagatagtggaaaaggaaggtggctcctacaaatgccatcattgcgataaaggaaaggccatcgttgaagatgcctctgccgacagtggtcccaaagatggacccccacccacgaggagcatcgtggaaaaagaagacgttccaaccacgtcttcaaagcaagtggattgatgtgatatctccactgacgtaagggatgacgcacaatcccactatccttcgcaagacccttcctctatataaggaagttcatttcatttggagagaacacgggggacgcgatcg

SEQ ID NO: 32 - DNA, 25 bp, synthetic construct
  source 1..25: mol_type = other DNA
gtttacaccacaatatatcctgcca

SEQ ID NO: 33 - DNA, 25 bp, synthetic construct
  source 1..25: mol_type = other DNA
gtttacccgccaatatatcctgtca

SEQ ID NO: 34 - DNA, 421 bp, synthetic construct
  source 1..421: mol_type = other DNA
cgacttgccttccgcacaatacatcatttcttcttagctttttttcttcttcttcgttcatacagtttttttttgtttatcagcttacattttcttgaaccgtagctttcgttttcttctttttaactttccattcggagtttttgtatcttgtttcatagtttgtcccaggattagaatgattaggcatcgaaccttcaagaatttgattgaataaaacatcttcattcttaagatatgaagataatcttcaaaaggcccctgggaatctgaaagaagagaagcaggcccatttatatgggaaagaacaatagtatttcttatataggcccatttaagttgaaaacaatcttcaaaagtcccacatcgcttagataagaaaacgaagctgagtttatatacagctagagtcgaagtagtg

SEQ ID NO: 35 - DNA, 20 bp, synthetic construct
  source 1..20: mol_type = other DNA
gtgatatctccactgacgta

SEQ ID NO: 36 - DNA, 20 bp, synthetic construct
  source 1..20: mol_type = other DNA
tgatatctccactgacgtaa

SEQ ID NO: 37 - DNA, 20 bp, synthetic construct
  source 1..20: mol_type = other DNA
tgcgtcatcccttacgtcag

SEQ ID NO: 38 - DNA, 76 bp, synthetic construct
  source 1..76: mol_type = other DNA
gttttagagctagaaatagcaagttaaaataaggctagtccgttatcaacttgaaaaagtggcaccgagtcggtgc

SEQ ID NO: 39 - DNA, 20 bp, synthetic construct
  source 1..20: mol_type = other DNA
tttttttgttttttatgtct

SEQ ID NO: 40 - DNA, 345 bp, synthetic construct
  source 1..345: mol_type = other DNA
tgagacttttcaacaaagggtaatatccggaaacctcctcggattccattgcccagctatctgtcactttattgtgaagatagtggaaaaggaaggtggctcctacaaatgccatcattgcgataaaggaaaggccatcgttgaagatgcctctgccgacagtggtcccaaagatggacccccacccacgaggagcatcgtggaaaaagaagacgttccaaccacgtcttcaaagcaagtggattgatgtgatatctccactgacgtaagggatgacgcacaatcccactatccttcgcaagacccttcctctatataaggaagttcatttcatttggagaggac

SEQ ID NO: 41 - DNA, 4101 bp, synthetic construct
  source 1..4101: mol_type = other DNA
gataagaagtactctatcggacttgccatcggaaccaactctgttggatgggctgttatcaccgatgagtacaaggttccatctaagaagttcaaggttcttggaaacaccgatagacactctatcaagaagaaccttatcggtgctcttcttttcgattctggagagaccgctgaggctaccagattgaagagaaccgctagaagaagatacaccagaagaaagaacagaatctgctaccttcaggaaatcttctctaacgagatggctaaggttgatgattctttcttccacagacttgaggagtctttccttgttgaggaggataagaagcacgagagacacccaatcttcggaaacatcgttgatgaggttgcttaccacgagaagtacccaaccatctaccaccttagaaagaagttggttgattctaccgataaggctgatcttagacttatctaccttgctcttgctcacatgatcaagttcagaggacacttccttatcgagggagaccttaacccagataactctgatgttgataagttgttcatccagcttgttcagacctacaaccagcttttcgaggagaacccaatcaacgcttctggagttgatgctaaggctatcctttctgctagactttctaagtctcgtagacttgagaaccttatcgctcagcttccaggagagaagaagaacggacttttcggaaaccttatcgctctttctcttggacttaccccaaacttcaagtctaacttcgatcttgctgaggatgctaagttgcagctttctaaggatacctacgatgatgatcttgataaccttcttgctcagatcggagatcagtacgctgatcttttccttgctgctaagaacctttctgatgctatccttctttctgacatccttagagttaacaccgagatcaccaaggctccactttctgcttctatgatcaagagatacgatgagcaccaccaggatcttacccttttgaaggctcttgttagacagcagcttccagagaagtacaaggaaatcttcttcgatcagtctaagaacggatacgctggatacatcgatggaggagcttctcaggaggagttctacaagttcatcaagccaatccttgagaagatggatggaaccgaggagcttcttgttaagttgaacagagaggatcttcttagaaagcagagaaccttcgataacggatctatcccacaccagatccaccttggagagcttcacgctatccttcgtagacaggaggatttctacccattcttgaaggataacagagagaagatcgagaagatccttaccttcagaatcccatactacgttggaccacttgctagaggaaactctcgtttcgcttggatgaccagaaagtctgaggagaccatcaccccttggaacttcgaggaggttgttgataagggagcttctgctcagtctttcatcgagagaatgaccaacttcgataagaaccttccaaacgagaaggttcttccaaagcactctcttctttacgagtacttcaccgtttacaacgagcttaccaaggttaagtacgttaccgagggaatgagaaagccagctttcctttctggagagcagaagaaggctatcgttgatcttcttttcaagaccaacagaaaggttaccgttaagcagttgaaggaggattacttcaagaagatcgagtgcttcgattctgttgaaatctctggagttgaggatagattcaacgcttctcttggaacctaccacgatcttttgaagatcatcaaggataaggatttccttgataacgaggagaacgaggacatccttgaggacatcgttcttacccttacccttttcgaggatagagagatgatcgaggagagactcaagacctacgctcaccttttcgatgataaggttatgaagcagttgaagagaagaagatacaccggatggggtagactttctcgtaagttgatcaacggaatcagagataagcagtctggaaagaccatccttgatttcttgaagtctgatggattcgctaacagaaacttcatgcagcttatccacgatgattctcttaccttcaaggaggacatccagaaggctcaggtttctggacagggagattctcttcacgagcacatcgctaaccttgctggatctccagctatcaagaagggaatccttcagaccgttaaggttgttgatgagcttgttaaggttatgggtagacacaagccagagaacatcgttatcgagatggctagagagaaccagaccacccagaagggacagaagaactctcgtgagagaatgaagagaatcgaggagggaatcaaggagcttggatctcaaatcttgaaggagcacccagttgagaacacccagcttcagaacgagaagttgtacctttactaccttcagaacggaagagatatgtacgttgatcaggagcttgacatcaacagactttctgattacgatgttgatgccatcgttccacagtctttcttgaaggatgattctatcgataacaaggttcttacccgttctgataagaacagaggaaagtctgataacgttccatctgaggaggttgttaagaagatgaagaactactggagacagcttcttaacgctaagttgatcacccagagaaagttcgataaccttaccaaggctgagagaggaggactttctgagcttgataaggctggattcatcaagagacagcttgttgagaccagacagatcaccaagcacgttgctcagatccttgattctcgtatgaacaccaagtacgatgagaacgataagttgatcagagaggttaaggttatcaccttgaagtctaagttggtttctgatttcagaaaggatttccagttctacaaggttagagagatcaacaactaccaccacgctcacgatgcttaccttaacgctgttgttggaaccgctcttatcaagaagtacccaaagttggagtctgagttcgtttacggagattacaaggtttacgatgttagaaagatgatcgctaagtctgagcaggagatcggaaaggctaccgctaagtacttcttctactctaacatcatgaacttcttcaagaccgagatcacccttgctaacggagagatcagaaagagaccacttatcgagaccaacggagagaccggagagatcgtttgggataagggaagagatttcgctaccgttagaaaggttctttctatgccacaggttaacatcgttaagaaaaccgaggttcagaccggaggattctctaaggagtctatccttccaaagagaaactctgataagttgatcgctagaaagaaggattgggacccaaagaagtacggaggattcgattctccaaccgttgcttactctgttcttgttgttgctaaggttgagaagggaaagtctaagaagttgaagtctgttaaggagcttcttggaatcaccatcatggagcgttcttctttcgagaagaacccaatcgatttccttgaggctaagggatacaaggaggttaagaaggatcttatcatcaagttgccaaagtactctcttttcgagcttgagaacggaagaaagagaatgcttgcttctgctggagagcttcagaagggaaacgagcttgctcttccatctaagtacgttaacttcctttaccttgcttctcactacgagaagttgaagggatctccagaggataacgagcagaagcagcttttcgttgagcagcacaagcactaccttgatgagatcatcgagcaaatctctgagttctctaagagagttatccttgctgatgctaaccttgataaggttctttctgcttacaacaagcacagagataagccaatcagagagcaggctgagaacatcatccaccttttcacccttaccaaccttggtgctccagctgctttcaagtacttcgataccaccatcgatagaaaaagatacacctctaccaaggaggttcttgatgctacccttatccaccagtctatcaccggactttacgagaccagaatcgatctttctcagcttggaggagat

SEQ ID NO: 42 - DNA, 189 bp, synthetic construct
  source 1..189: mol_type = other DNA
gtaagtttctgcttctacctttgatatatatataataattatcattaattagtagtaatataatatttcaaatatttttttcaaaataaaagaatgtagtatatagcaattgcttttctgtagtttataagtgtgtatattttaatttataacttttctaatatatgaccaaaatttgttgatgtgcag

SEQ ID NO: 43 - DNA, 48 bp, synthetic construct
  source 1..48: mol_type = other DNA
gattacaaggatgatgatgataaggattacaaggatgatgatgataag

SEQ ID NO: 44 - DNA, 48 bp, synthetic construct
  source 1..48: mol_type = other DNA
aagagaccagctgctaccaagaaggctggacaggctaagaagaagaag

SEQ ID NO: 45 - DNA, 54 bp, synthetic construct
  source 1..54: mol_type = other DNA
gagggcagaggaagtcttctaacatgcggtgacgtggaggagaatcccggccct

SEQ ID NO: 46 - DNA, 351 bp, synthetic construct
  source 1..351: mol_type = other DNA
atggcttctaactttactcagttcgttctcgtcgacaatggcggaactggcgacgtgactgtcgccccaagcaacttcgctaacgggatcgctgaatggatcagctctaactcgcgttcacaggcttacaaagtaacctgtagcgttcgtcagagctctgcgcagaatcgcaaatacaccatcaaagtcgaggtgcctaaaggcgcctggcgttcgtacttaaatatggaactaaccattccaattttcgccacgaattccgactgcgagcttattgttaaggcaatgcaaggtctcctaaaagatggaaacccgattccctcagcaatcgcagcaaactccggcatctac

SEQ ID NO: 47 - DNA, 1326 bp, synthetic construct
  source 1..1326: mol_type = other DNA
ctgttggatccgggaacacctatggacgctgatttggtagcttcttctacagtagtgtgggaacaagatgcagatccttttgctggaacagccgacgacttccccgccttcaatgaagaggagcttgcatggttgatggagctgttacctcaaggaggatcagggggtcttttagatccaggtactcccatggatgcagacctggtcgcttcaagtacagtcgtttgggagcaggatgctgatccattcgcaggtacagcagatgacttcccggctttcaatgaggaggaacttgcttggctcatggaattgctcccgcaggcaagaggtggatctggtggtctgctcgacccaggaacgccgatggacgctgatctggtagcatctagtacagtctgggagcaggacgctgacccattcgctggtacggctgacgattttcctgcctttaatgaggaagagttagcctggctgatggagttattaccccagggcggtagtggcggattattggaccctggtacgccgatggatgcagaccttgtggcttcatcaacggtcgtatgggagcaggatgccgatcctttcgcaggaaccgcagacgacttcccagcctttaacgaagaagagctcgcatggcttatggaacttttacctcaggcacgtggaggaagtggtgggctcctggatccaggcactccgatggacgcagacttagtagctagttccaccgttgtctgggagcaggatgcagatccttttgctggtaccgcagacgacttccctgctttcaatgaagaagaattggcctggcttatggaattacttccgcagggtgggtctggtgggctgctcgatcccggtacgccgatggatgctgacttggttgctagcagtactgtggtctgggaacaggatgctgaccccttcgctgggactgccgacgacttcccagccttcaacgaagaggaactcgcatggttgatggaactgcttcctcaagcacgtggggggtcaggcggaggcggatctggcggtgacgcactggacgactttgatctcgacatgcttgggtccgatgctctcgacgattttgacctcgatatgcttgggtctgacgcattagatgactttgatttagacatgttggggtcagacgctttggacgatttcgacttagatatgttggccagaggtagtgatgctcttgacgattttgacctcgatatgctcgacgctcttgatgattttgatctcgacatgctcgatgcacttgatgactttgaccttgacatgctcgacgcactcgatgacttcgacctcgac

SEQ ID NO: 48 - DNA, 253 bp, synthetic construct; identical to SEQ ID NO: 22
  source 1..253: mol_type = other DNA

SEQ ID NO: 49 - DNA, 810 bp, synthetic construct
  source 1..810: mol_type = other DNA
ttagaaaaactcatcgagcatcaaatgaaactgcaatttattcatatcaggattatcaataccatatttttgaaaaagccgtttctgtaatgaaggagaaaactcaccgaggcagttccataggatggcaagatcctggtatcggtctgcgattccgactcgtccaacatcaatacaacctattaatttcccctcgtcaaaaataaggttatcaagtgagaaatcaccatgagtgacgactgaatccggtgagaatggcaaaagtttatgcatttctttccagacttgttcaacaggccagccattacgctcgtcatcaaaatcactcgcatcaaccaaaccgttattcattcgtgattgcgcctgagcgagacgaaatacgcgatcgctgttaaaaggacaattacaaacaggaatcgaatgcaaccggcgcagggacactgccagcgcatcaacaatattttcacctgaatcaggatattcttctaatacctggaatgctgtttttccggggatcgcagtggtgagtaaccatgcatcatcaggagtacggataaaatgcttgatggtcggaagaggcataaattccgtcagccagtttagtctgaccatctcatctgtaacatcattggcaacgctacctttgccatgtttcagaaacaactctggcgcatcgggcttcccatacaagcgatagattgtcgcacctgattgcccgacattatcgcgagcccatttatacccatataaatcagcatccatgttggaatttaatcgcggcctcgacgtttcccgttgaatatggctcat

SEQ ID NO: 50 - DNA, 11387 bp, synthetic construct
  source 1..11387: mol_type = other DNA
ttctaataaacgctcttttctcttaggtttacccgccaatatatcctgtcaaacactgatagtttaaactgaaggcgggaaacgacaatctgatccaagctcaagctaagctcacgtgacggaattaagcttcgacttgccttccgcacaatacatcatttcttcttagctttttttcttcttcttcgttcatacagtttttttttgtttatcagcttacattttcttgaaccgtagctttcgttttcttctttttaactttccattcggagtttttgtatcttgtttcatagtttgtcccaggattagaatgattaggcatcgaaccttcaagaatttgattgaataaaacatcttcattcttaagatatgaagataatcttcaaaaggcccctgggaatctgaaagaagagaagcaggcccatttatatgggaaagaacaatagtatttcttatataggcccatttaagttgaaaacaatcttcaaaagtcccacatcgcttagataagaaaacgaagctgagtttatatacagctagagtcgaagtagtggtgatatctccactgacgtagtttaagagctatgctggaaacagcatagcaagtttaaataaggctagtccgttatcaacttgaaaaagtggcaccgagtcggtgcgggagcacatgaggatcacccatgtgcgactcccacagtcactggggagtcttccctttttttgttttttatgtctagatcgatttcttcttcctctgttcttcggcgttcaatttctggggttttctcttcgttttctgtaactgaaacctaaaatttgacctaaaaaaaatctcaaataatatgattcagtggttttgtacttttcagttagttgagttttgcagttccgatgagataaaccaataagcttgcatgcctgcaggtcaacatggtggagcacgacacacttgtctactccaaaaatatcaaagatacagtctcagaagaccaaagggcaattgagacttttcaacaaagggtaatatccggaaacctcctcggattccattgcccagctatctgtcactttattgtgaagatagtggaaaaggaaggtggctcctacaaatgccatcattgcgataaaggaaaggccatcgttgaagatgcctctgccgacagtggtcccaaagatggacccccacccacgaggagcatcgtggaaaaagaagacgttccaaccacgtcttcaaagcaagtggattgatgtgataacatggtggagcacgacacacttgtctactccaaaaatatcaaagatacagtctcagaagaccaaagggcaattgagacttttcaacaaagggtaatatccggaaacctcctcggattccattgcccagctatctgtcactttattgtgaagatagtggaaaaggaaggtggctcctacaaatgccatcattgcgataaaggaaaggccatcgttgaagatgcctctgccgacagtggtcccaaagatggacccccacccacgaggagcatcgtggaaaaagaagacgttccaaccacgtcttcaaagcaagtggattgatgtgatatctccactgacgtaagggatgacgcacaatcccactatccttcgcaagacccttcctctatataaggaagttcatttcatttggagaggacctcgacctcaacacaacatatacaaaacaaacgaatctcaagcaatcaagcattctacttctattgcagcaatttaaatcatttcttttaaagcaaaagcaattttctgaaaattttcaccatttacgaacgatactcgagggggatccccaatacttgtatggccgcggccgctctagatggattacaaggatgatgatgataaggattacaaggatgatgatgataagatggctccaaagaagaagagaaaggttggaatccacggagttccagctgctgataagaagtactctatcggacttgccatcggaaccaactctgttggatgggctgttatcaccgatgagtacaaggttccatctaagaagttcaaggttcttggaaacaccgatagacactctatcaagaagaaccttatcggtgctcttcttttcgattctggagagaccgctgaggctaccagattgaagagaaccgctagaagaagatacaccagaagaaagaacagaatctgctaccttcaggaaatcttctctaacgagatggctaaggttgatgattctttcttccacagacttgaggagtctttccttgttgaggaggataagaagcacgagagacacccaatcttcggaaacatcgttgatgaggttgcttaccacgagaagtacccaaccatctaccaccttagaaagaagttggttgattctaccgataaggctgatcttagacttatctaccttgctcttgctcacatgatcaagttcagaggacacttccttatcgagggagaccttaacccagataactctgatgttgataagttgttcatccagcttgttcagacctacaaccagcttttcgaggagaacccaatcaacgcttctggagttgatgctaaggctatcctttctgctagactttctaagtctcgtagacttgagaaccttatcgctcagcttccaggagagaagaagaacggacttttcggaaaccttatcgctctttctcttggacttaccccaaacttcaagtctaacttcgatcttgctgaggatgctaagttgcagctttctaaggatacctacgatgatgatcttgataaccttcttgctcagatcggagatcagtacgctgatcttttccttgctgctaagaacctttctgatgctatccttctttctgacatccttagagttaacaccgagatcaccaaggctccactttctgcttctatgatcaagagatacgatgagcaccaccaggatcttacccttttgaaggctcttgttagacagcagcttccagagaagtacaaggaaatcttcttcgatcagtctaagaacggatacgctggatacatcgatggaggagcttctcaggaggagttctacaagttcatcaagccaatccttgagaagatggatggaaccgaggagcttcttgttaagttgaacagagaggatcttcttagaaagcagagaaccttcgataacggatctatcccacaccagatccaccttggagagcttcacgctatccttcgtagacaggaggatttctacccattcttgaaggataacagagagaagatcgagaagatccttaccttcagaatcccatactacgttggaccacttgctagaggaaactctcgtttcgcttggatgaccagaaagtctgaggagaccatcaccccttggaacttcgaggaggtaagtttctgcttctacctttgatatatatataataattatcattaattagtagtaatataatatttcaaatatttttttcaaaataaaagaatgtagtatatagcaattgcttttctgtagtttataagtgtgtatattttaatttataacttttctaatatatgaccaaaatttgttgatgtgcaggttgttgataagggagcttctgctcagtctttcatcgagagaatgaccaacttcgataagaaccttccaaacgagaaggttcttccaaagcactctcttctttacgagtacttcaccgtttacaacgagcttaccaaggttaagtacgttaccgagggaatgagaaagccagctttcctttctggagagcagaagaaggctatcgttgatcttcttttcaagaccaacagaaaggttaccgttaagcagttgaaggaggattacttcaagaagatcgagtgcttcgattctgttgaaatctctggagttgaggatagattcaacgcttctcttggaacctaccacgatcttttgaagatcatcaaggataaggatttccttgataacgaggagaacgaggacatccttgaggacatcgttcttacccttacccttttcgaggatagagagatgatcgaggagagactcaagacctacgctcaccttttcgatgataaggttatgaagcagttgaagagaagaagatacaccggatggggtagactttctcgtaagttgatcaacggaatcagagataagcagtctggaaagaccatccttgatttcttgaagtctgatggattcgctaacagaaacttcatgcagcttatccacgatgattctcttaccttcaaggaggacatccagaaggctcaggtttctggacagggagattctcttcacgagcacatcgctaaccttgctggatctccagctatcaagaagggaatccttcagaccgttaaggttgttgatgagcttgttaaggttatgggtagacacaagccagagaacatcgttatcgagatggctagagagaaccagaccacccagaagggacagaagaactctcgtgagagaatgaagagaatcgaggagggaatcaaggagcttggatctcaaatcttgaaggagcacccagttgagaacacccagcttcagaacgagaagttgtacctttactaccttcagaacggaagagatatgtacgttgatcaggagcttgacatcaacagactttctgattacgatgttgatgccatcgttccacagtctttcttgaaggatgattctatcgataacaaggttcttacccgttctgataagaacagaggaaagtctgataacgttccatctgaggaggttgttaagaagatgaagaactactggagacagcttcttaacgctaagttgatcacccagagaaagttcgataaccttaccaaggctgagagaggaggactttctgagcttgataaggctggattcatcaagagacagcttgttgagaccagacagatcaccaagcacgttgctcagatccttgattctcgtatgaacaccaagtacgatgagaacgataagttgatcagagaggttaaggttatcaccttgaagtctaagttggtttctgatttcagaaaggatttccagttctacaaggttagagagatcaacaactaccaccacgctcacgatgcttaccttaacgctgttgttggaaccgctcttatcaagaagtacccaaagttggagtctgagttcgtttacggagattacaaggtttacgatgttagaaagatgatcgctaagtctgagcaggagatcggaaaggctaccgctaagtacttcttctactctaacatcatgaacttcttcaagaccgagatcacccttgctaacggagagatcagaaagagaccacttatcgagaccaacggagagaccggagagatcgtttgggataagggaagagatttcgctaccgttagaaaggttctttctatgccacaggttaacatcgttaagaaaaccgaggttcagaccggaggattctctaaggagtctatccttccaaagagaaactctgataagttgatcgctagaaagaaggattgggacccaaagaagtacggaggattcgattctccaaccgttgcttactctgttcttgttgttgctaaggttgagaagggaaagtctaagaagttgaagtctgttaaggagcttcttggaatcaccatcatggagcgttcttctttcgagaagaacccaatcgatttccttgaggctaagggatacaaggaggttaagaaggatcttatcatcaagttgccaaagtactctcttttcgagcttgagaacggaagaaagagaatgcttgcttctgctggagagcttcagaagggaaacgagcttgctcttccatctaagtacgttaacttcctttaccttgcttctcactacgagaagttgaagggatctccagaggataacgagcagaagcagcttttcgttgagcagcacaagcactaccttgatgagatcatcgagcaaatctctgagttctctaagagagttatccttgctgatgctaaccttgataaggttctttctgcttacaacaagcacagagataagccaatcagagagcaggctgagaacatcatccaccttttcacccttaccaaccttggtgctccagctgctttcaagtacttcgataccaccatcgatagaaaaagatacacctctaccaaggaggttcttgatgctacccttatccaccagtctatcaccggactttacgagaccagaatcgatctttctcagcttggaggagataagagaccagctgctaccaagaaggctggacaggctaagaagaagaaggagggcagaggaagtcttctaacatgcggtgacgtggaggagaatcccggccctatgatggcttctaactttactcagttcgttctcgtcgacaatggcggaactggcgacgtgactgtcgccccaagcaacttcgctaacgggatcgctgaatggatcagctctaactcgcgttcacaggcttacaaagtaacctgtagcgttcgtcagagctctgcgcagaatcgcaaatacaccatcaaagtcgaggtgcctaaaggcgcctggcgttcgtacttaaatatggaactaaccattccaattttcgccacgaattccgactgcgagcttattgttaaggcaatgcaaggtctcctaaaagatggaaacccgattccctcagcaatcgcagcaaactccggcatctaccctaagaagaagaggaaggttctgttggatccgggaacacctatggacgctgatttggtagcttcttctacagtagtgtgggaacaagatgcagatccttttgctggaacagccgacgacttccccgccttcaatgaagaggagcttgcatggttgatggagctgttacctcaaggaggatcagggggtcttttagatccaggtactcccatggatgcagacctggtcgcttcaagtacagtcgtttgggagcaggatgctgatccattcgcaggtacagcagatgacttcccggctttcaatgaggaggaacttgcttggctcatggaattgctcccgcaggcaagaggtggatctggtggtctgctcgacccaggaacgccgatggacgctgatctggtagcatctagtacagtctgggagcaggacgctgacccattcgctggtacggctgacgattttcctgcctttaatgaggaagagttagcctggctgatggagttattaccccagggcggtagtggcggattattggaccctggtacgccgatggatgcagaccttgtggcttcatcaacggtcgtatgggagcaggatgccgatcctttcgcaggaaccgcagacgacttcccagcctttaacgaagaagagctcgcatggcttatggaacttttacctcaggcacgtggaggaagtggtgggctcctggatccaggcactccgatggacgcagacttagtagctagttccaccgttgtctgggagcaggatgcagatccttttgctggtaccgcagacgacttccctgctttcaatgaagaagaattggcctggcttatggaattacttccgcagggtgggtctggtgggctgctcgatcccggtacgccgatggatgctgacttggttgctagcagtactgtggtctgggaacaggatgctgaccccttcgctgggactgccgacgacttcccagccttcaacgaagaggaactcgcatggttgatggaactgcttcctcaagcacgtggggggtcaggcggaggcggatctggcggtgacgcactggacgactttgatctcgacatgcttgggtccgatgctctcgacgattttgacctcgatatgcttgggtctgacgcattagatgactttgatttagacatgttggggtcagacgctttggacgatttcgacttagatatgttggccagaggtagtgatgctcttgacgattttgacctcgatatgctcgacgctcttgatgattttgatctcgacatgctcgatgcacttgatgactttgaccttgacatgctcgacgcactcgatgacttcgacctcgacatgcttaagctttgagctcaggcctccatacaagtattggggatccactacgaatttccccgatcgttcaaacatttggcaataaagtttcttaagattgaatcctgttgccggtcttgcgatgattatcatataatttctgttgaattacgttaagcatgtaataattaacatgtaatgcatgacgttatttatgagatgggtttttatgattagagtcccgcaattatacatttaatacgcgatagaaaacaaaatatagcgcgcaaactaggataaattatcgcgcgcggtgtcatctatgttactagatcgggctagtcaggttaactcaattcggcgttaattcagtacattaaaaacgtccgcaatgtgttattaagttgtctaagcgtcaatttgtttacaccacaatatatcctgccaccagccagccaacagctccccgaccggcagctcggcacaaaatcaccactcgatacaggcagcccatcagtccgggacggcgtcagcgggagagccgttgtaaggcggcagactttgctcatgttaccgatgctattcggaagaacggcaactaagctgccgggtttgaaacacggatgatctcgcggagggtagcatgttgattgtaacgatgacagagcgttgctgcctgtgatcacttaagtaactaactaacaggaagagtttgtagaaacgcaaaaaggccatccgtcaggatggccttctgcttagtttgatgcctggcagtttatggcgggcgtcctgcccgccaccctccgggccgttgcttcacaacgttcaaatccgctcccggcggatttgtcctactcaggagagcgttcaccgacaaacaacagataaaacgaaaggcccagtcttccgactgagcctttcgttttatttgatgcctggcagttccctactctcgcttagtagttagacgtccccgagatccatgctagaccatgaatccagaagcccgagaggttgccgcctttcgggctttttctttttcaaaaaaaaaaatttataaaacgatctgttgcggccggccgccgggttgtgggcaaaggcgctcgacggtgggcaaccgcttgcggttgtccacgggcggagccggtgcgcgtagcgcattgtccacaagccaagggcgaccaataattgatatatatattcataattgaaaagctaattgaacatactacttgctgtaactacttgccggagcgaggggtgtttgcaagctgttgatctgaaagggctattagcgttctcacgtgcctttttgattagcgatttcacgtgaccttattagcgatttcacgtactccgattagcgatttcacgtaccctgattagcgatttcacgtggatagtttttggagcgggccggaaagccccgtgaatcaaggctttgcggggcattagcggtttcacgtggataactaccctctatccacaggcttccggggataaaaaagcccgctcgacggcgggctgttggatggggatctagcggtaatacggttatccacagaatcaggggataacgcaggaaagaacatgtgagcaaaaggccagcaaaaggccaggaaccgtaaaaaggccgcgttgctggcgtttttccataggctccgcccccctgacgagcatcacaaaaatcgacgctcaagtcagaggtggcgaaacccgacaggactataaagataccaggcgtttccccctggaagctccctcgtgcgctctcctgttccgaccctgccgcttaccggatacctgtccgcctttctcccttcgggaagcgtggcgctttctcatagctcacgctgtaggtatctcagttcggtgtaggtcgttcgctccaagctgggctgtgtgcacgaaccccccgttcagcccgaccgctgcgccttatccggtaactatcgtcttgagtccaacccggtaagacacgacttatcgccactggcagcagccactggtaacaggattagcagagcgaggtatgtaggcggtgctacagagttcttgaagtggtggcctaactacggctacactagaagaacagtatttggtatctgcgctctgctgaagccagttaccttcggaaaaagagttggtagctcttgatccggcaaacaaaccaccgctggtagcggtggtttttttgtttgcaagcagcagattacgcgcagaaaaaaaggatctcaagaagatcctttgatcttttctacggggtctgacgctcagtggaacggggcccaatctgaataatgttacaaccaattaaccaattctgattagaaaaactcatcgagcatcaaatgaaactgcaatttattcatatcaggattatcaataccatatttttgaaaaagccgtttctgtaatgaaggagaaaactcaccgaggcagttccataggatggcaagatcctggtatcggtctgcgattccgactcgtccaacatcaatacaacctattaatttcccctcgtcaaaaataaggttatcaagtgagaaatcaccatgagtgacgactgaatccggtgagaatggcaaaagtttatgcatttctttccagacttgttcaacaggccagccattacgctcgtcatcaaaatcactcgcatcaaccaaaccgttattcattcgtgattgcgcctgagcgagacgaaatacgcgatcgctgttaaaaggacaattacaaacaggaatcgaatgcaaccggcgcagggacactgccagcgcatcaacaatattttcacctgaatcaggatattcttctaatacctggaatgctgtttttccggggatcgcagtggtgagtaaccatgcatcatcaggagtacggataaaatgcttgatggtcggaagaggcataaattccgtcagccagtttagtctgaccatctcatctgtaacatcattggcaacgctacctttgccatgtttcagaaacaactctggcgcatcgggcttcccatacaagcgatagattgtcgcacctgatccggtactagaggaactgaaattgcccgacattatcgcgagcccatttatacccatataaatcagcatccatgttggaatttaatcgcggcctcgacgtttcccgttgaatatggctcataacaccccttgtattactgtttatgtaagcagacagttttattgttcatgatgatatatttttatcttgtgcaatgtaacatcagagattttgagacacgggccagagctgcagtttgatcccgaggggaaccctgtggttgacatgcacatacaaatggacgaacggataaaccttttcacgcccttttaaatatccgtta

SEQ ID NO: 51 - DNA, 186 bp, synthetic construct
  source 1..186: mol_type = other DNA
cggacactggtgaccttcaaggatgtatttgtggacttcaccagggaggagtggaagctgctggacactgctcagcagatcgtgtacagaaatgtgatgctggagaactataagaacctggtttccttgggttatcagcttactaagccagatgtgatcctccggttggagaagggagaagagccc

SEQ ID NO: 52 - DNA, 20 bp, synthetic construct
  source 1..20: mol_type = other DNA
tagctattgaaatttggata

SEQ ID NO: 53 - DNA, 20 bp, synthetic construct
  source 1..20: mol_type = other DNA
ttttggatttgctacattgt

SEQ ID NO: 54 - DNA, 20 bp, synthetic construct
  source 1..20: mol_type = other DNA
tatgttttgagaagcattta

SEQ ID NO: 55 - DNA, 10101 bp, synthetic construct
  source 1..10101: mol_type = other DNA
cgctcttttctcttaggtttacccgccaatatatcctgtcaaacactgatagtttaaactgaaggcgggaaacgacaatctgatccaagctcaagctaagctcacgtgacggaattaagcttcgacttgccttccgcacaatacatcatttcttcttagctttttttcttcttcttcgttcatacagtttttttttgtttatcagcttacattttcttgaaccgtagctttcgttttcttctttttaactttccattcggagtttttgtatcttgtttcatagtttgtcccaggattagaatgattaggcatcgaaccttcaagaatttgattgaataaaacatcttcattcttaagatatgaagataatcttcaaaaggcccctgggaatctgaaagaagagaagcaggcccatttatatgggaaagaacaatagtatttcttatataggcccatttaagttgaaaacaatcttcaaaagtcccacatcgcttagataagaaaacgaagctgagtttatatacagctagagtcgaagtagtgtagctattgaaatttggatagtttaagagctatgctggaaacagcatagcaagtttaaataaggctagtccgttatcaacttgaaaaagtggcaccgagtcggtgcctgaatgcctgcgagcatctttttttgttttttatgtctagatcgatttcttcttcctctgttcttcggcgttcaatttctggggttttctcttcgttttctgtaactgaaacctaaaatttgacctaaaaaaaatctcaaataatatgattcagtggttttgtacttttcagttagttgagttttgcagttccgatgagataaaccaataagcttgcatgcctgcaggtcaacatggtggagcacgacacacttgtctactccaaaaatatcaaagatacagtctcagaagaccaaagggcaattgagacttttcaacaaagggtaatatccggaaacctcctcggattccattgcccagctatctgtcactttattgtgaagatagtggaaaaggaaggtggctcctacaaatgccatcattgcgataaaggaaaggccatcgttgaagatgcctctgccgacagtggtcccaaagatggacccccacccacgaggagcatcgtggaaaaagaagacgttccaaccacgtcttcaaagcaagtggattgatgtgataacatggtggagcacgacacacttgtctactccaaaaatatcaaagatacagtctcagaagaccaaagggcaattgagacttttcaacaaagggtaatatccggaaacctcctcggattccattgcccagctatctgtcactttattgtgaagatagtggaaaaggaaggtggctcctacaaatgccatcattgcgataaaggaaaggccatcgttgaagatgcctctgccgacagtggtcccaaagatggacccccacccacgaggagcatcgtggaaaaagaagacgttccaaccacgtcttcaaagcaagtggattgatgtgatatctccactgacgtaagggatgacgcacaatcccactatccttcgcaagacccttcctctatataaggaagttcatttcatttggagaggacctcgacctcaacacaacatatacaaaacaaacgaatctcaagcaatcaagcattctacttctattgcagcaatttaaatcatttcttttaaagcaaaagcaattttctgaaaattttcaccatttacgaacgatactcgagggggatccccaatacttgtatggccgcggccgctctagatggattacaaggatgatgatgataaggattacaaggatgatgatgataagatggctccaaagaagaagagaaaggttggaatccacggagttccagctgctgataagaagtactctatcggacttgccatcggaaccaactctgttggatgggctgttatcaccgatgagtacaaggttccatctaagaagttcaaggttcttggaaacaccgatagacactctatcaagaagaaccttatcggtgctcttcttttcgattctggagagaccgctgaggctaccagattgaagagaaccgctagaagaagatacaccagaagaaagaacagaatctgctaccttcaggaaatcttctctaacgagatggctaaggttgatgattctttcttccacagacttgaggagtctttccttgttgaggaggataagaagcacgagagacacccaatcttcggaaacatcgttgatgaggttgcttaccacgagaagtacccaaccatctaccaccttagaaagaagttggttgattctaccgataaggctgatcttagacttatctaccttgctcttgctcacatgatcaagttcagaggacacttccttatcgagggagaccttaacccagataactctgatgttgataagttgttcatccagcttgttcagacctacaaccagcttttcgaggagaacccaatcaacgcttctggagttgatgctaaggctatcctttctgctagactttctaagtctcgtagacttgagaaccttatcgctcagcttccaggagagaagaagaacggacttttcggaaaccttatcgctctttctcttggacttaccccaaacttcaagtctaacttcgatcttgctgaggatgctaagttgcagctttctaaggatacctacgatgatgatcttgataaccttcttgctcagatcggagatcagtacgctgatcttttccttgctgctaagaacctttctgatgctatccttctttctgacatccttagagttaacaccgagatcaccaaggctccactttctgcttctatgatcaagagatacgatgagcaccaccaggatcttacccttttgaaggctcttgttagacagcagcttccagagaagtacaaggaaatcttcttcgatcagtctaagaacggatacgctggatacatcgatggaggagcttctcaggaggagttctacaagttcatcaagccaatccttgagaagatggatggaaccgaggagcttcttgttaagttgaacagagaggatcttcttagaaagcagagaaccttcgataacggatctatcccacaccagatccaccttggagagcttcacgctatccttcgtagacaggaggatttctacccattcttgaaggataacagagagaagatcgagaagatccttaccttcagaatcccatactacgttggaccacttgctagaggaaactctcgtttcgcttggatgaccagaaagtctgaggagaccatcaccccttggaacttcgaggaggtaagtttctgcttctacctttgatatatatataataattatcattaattagtagtaatataatatttcaaatatttttttcaaaataaaagaatgtagtatatagcaattgcttttctgtagtttataagtgtgtatattttaatttataacttttctaatatatgaccaaaatttgttgatgtgcaggttgttgataagggagcttctgctcagtctttcatcgagagaatgaccaacttcgataagaaccttccaaacgagaaggttcttccaaagcactctcttctttacgagtacttcaccgtttacaacgagcttaccaaggttaagtacgttaccgagggaatgagaaagccagctttcctttctggagagcagaagaaggctatcgttgatcttcttttcaagaccaacagaaaggttaccgttaagcagttgaaggaggattacttcaagaagatcgagtgcttcgattctgttgaaatctctggagttgaggatagattcaacgcttctcttggaacctaccacgatcttttgaagatcatcaaggataaggatttccttgataacgaggagaacgaggacatccttgaggacatcgttcttacccttacccttttcgaggatagagagatgatcgaggagagactcaagacctacgctcaccttttcgatgataaggttatgaagcagttgaagagaagaagatacaccggatggggtagactttctcgtaagttgatcaacggaatcagagataagcagtctggaaagaccatccttgatttcttgaagtctgatggattcgctaacagaaacttcatgcagcttatccacgatgattctcttaccttcaaggaggacatccagaaggctcaggtttctggacagggagattctcttcacgagcacatcgctaaccttgctggatctccagctatcaagaagggaatccttcagaccgttaaggttgttgatgagcttgttaaggttatgggtagacacaagccagagaacatcgttatcgagatggctagagagaaccagaccacccagaagggacagaagaactctcgtgagagaatgaagagaatcgaggagggaatcaaggagcttggatctcaaatcttgaaggagcacccagttgagaacacccagcttcagaacgagaagttgtacctttactaccttcagaacggaagagatatgtacgttgatcaggagcttgacatcaacagactttctgattacgatgttgatgccatcgttccacagtctttcttgaaggatgattctatcgataacaaggttcttacccgttctgataagaacagaggaaagtctgataacgttccatctgaggaggttgttaagaagatgaagaactactggagacagcttcttaacgctaagttgatcacccagagaaagttcgataaccttaccaaggctgagagaggaggactttctgagcttgataaggctggattcatcaagagacagcttgttgagaccagacagatcaccaagcacgttgctcagatccttgattctcgtatgaacaccaagtacgatgagaacgataagttgatcagagaggttaaggttatcaccttgaagtctaagttggtttctgatttcagaaaggatttccagttctacaaggttagagagatcaacaactaccaccacgctcacgatgcttaccttaacgctgttgttggaaccgctcttatcaagaagtacccaaagttggagtctgagttcgtttacggagattacaaggtttacgatgttagaaagatgatcgctaagtctgagcaggagatcggaaaggctaccgctaagtacttcttctactctaacatcatgaacttcttcaagaccgagatcacccttgctaacggagagatcagaaagagaccacttatcgagaccaacggagagaccggagagatcgtttgggataagggaagagatttcgctaccgttagaaaggttctttctatgccacaggttaacatcgttaagaaaaccgaggttcagaccggaggattctctaaggagtctatccttccaaagagaaactctgataagttgatcgctagaaagaaggattgggacccaaagaagtacggaggattcgattctccaaccgttgcttactctgttcttgttgttgctaaggttgagaagggaaagtctaagaagttgaagtctgttaaggagcttcttggaatcaccatcatggagcgttcttctttcgagaagaacccaatcgatttccttgaggctaagggatacaaggaggttaagaaggatcttatcatcaagttgccaaagtactctcttttcgagcttgagaacggaagaaagagaatgcttgcttctgctggagagcttcagaagggaaacgagcttgctcttccatctaagtacgttaacttcctttaccttgcttctcactacgagaagttgaagggatctccagaggataacgagcagaagcagcttttcgttgagcagcacaagcactaccttgatgagatcatcgagcaaatctctgagttctctaagagagttatccttgctgatgctaaccttgataaggttctttctgcttacaacaagcacagagataagccaatcagagagcaggctgagaacatcatccaccttttcacccttaccaaccttggtgctccagctgctttcaagtacttcgataccaccatcgatagaaaaagatacacctctaccaaggaggttcttgatgctacccttatccaccagtctatcaccggactttacgagaccagaatcgatctttctcagcttggaggagataagagaccagctgctaccaagaaggctggacaggctaagaagaagaaggagggcagaggaagtcttctaacatgcggtgacgtggaggagaatcccggccctatgcccaaaaagaaaagaaaagtgggtagtatgaaatcaattcgctgtaaaaactgcaacaaactgttatttaaggcggatagttttgatcacattgaaatcaggtgtccgcgttgcaaacgtcacatcataatgctgaatgcctgcgagcatcccacggagaaacattgtgggaaaagagaaaaaatcacgcattctgacgaaaccgtgcgttatggctccactagtgggcacaagcttaatggcggtggcggagggatggatgctaagtcactaactgcctggtcccggacactggtgaccttcaaggatgtatttgtggacttcaccagggaggagtggaagctgctggacactgctcagcagatcgtgtacagaaatgtgatgctggagaactataagaacctggtttccttgggttatcagcttactaagccagatgtgatcctccggttggagaagggagaagagcccatgcttaagctttgagctcaggcctccatacaagtattggggatccactacgaatttccccgatcgttcaaacatttggcaataaagtttcttaagattgaatcctgttgccggtcttgcgatgattatcatataatttctgttgaattacgttaagcatgtaataattaacatgtaatgcatgacgttatttatgagatgggtttttatgattagagtcccgcaattatacatttaatacgcgatagaaaacaaaatatagcgcgcaaactaggataaattatcgcgcgcggtgtcatctatgttactagatcgggctagtcaggttaactcaattcggcgttaattcagtacattaaaaacgtccgcaatgtgttattaagttgtctaagcgtcaatttgtttacaccacaatatatcctgccaccagccagccaacagctccccgaccggcagctcggcacaaaatcaccactcgatacaggcagcccatcagtccgggacggcgtcagcgggagagccgttgtaaggcggcagactttgctcatgttaccgatgctattcggaagaacggcaactaagctgccgggtttgaaacacggatgatctcgcggagggtagcatgttgattgtaacgatgacagagcgttgctgcctgtgatcacttaagtaactaactaacaggaagagtttgtagaaacgcaaaaaggccatccgtcaggatggccttctgcttagtttgatgcctggcagtttatggcgggcgtcctgcccgccaccctccgggccgttgcttcacaacgttcaaatccgctcccggcggatttgtcctactcaggagagcgttcaccgacaaacaacagataaaacgaaaggcccagtcttccgactgagcctttcgttttatttgatgcctggcagttccctactctcgcttagtagttagacgtccccgagatccatgctagaccatgaatccagaagcccgagaggttgccgcctttcgggctttttctttttcaaaaaaaaaaatttataaaacgatctgttgcggccggccgccgggttgtgggcaaaggcgctcgacggtgggcaaccgcttgcggttgtccacgggcggagccggtgcgcgtagcgcattgtccacaagccaagggcgaccaataattgatatatatattcataattgaaaagctaattgaacatactacttgctgtaactacttgccggagcgaggggtgtttgcaagctgttgatctgaaagggctattagcgttctcacgtgcctttttgattagcgatttcacgtgaccttattagcgatttcacgtactccgattagcgatttcacgtaccctgattagcgatttcacgtggatagtttttggagcgggccggaaagccccgtgaatcaaggctttgcggggcattagcggtttcacgtggataactaccctctatccacaggcttccggggataaaaaagcccgctcgacggcgggctgttggatggggatctagcggtaatacggttatccacagaatcaggggataacgcaggaaagaacatgtgagcaaaaggccagcaaaaggccaggaaccgtaaaaaggccgcgttgctggcgtttttccataggctccgcccccctgacgagcatcacaaaaatcgacgctcaagtcagaggtggcgaaacccgacaggactataaagataccaggcgtttccccctggaagctccctcgtgcgctctcctgttccgaccctgccgcttaccggatacctgtccgcctttctcccttcgggaagcgtggcgctttctcatagctcacgctgtaggtatctcagttcggtgtaggtcgttcgctccaagctgggctgtgtgcacgaaccccccgttcagcccgaccgctgcgccttatccggtaactatcgtcttgagtccaacccggtaagacacgacttatcgccactggcagcagccactggtaacaggattagcagagcgaggtatgtaggcggtgctacagagttcttgaagtggtggcctaactacggctacactagaagaacagtatttggtatctgcgctctgctgaagccagttaccttcggaaaaagagttggtagctcttgatccggcaaacaaaccaccgctggtagcggtggtttttttgtttgcaagcagcagattacgcgcagaaaaaaaggatctcaagaagatcctttgatcttttctacggggtctgacgctcagtggaacggggcccaatctgaataatgttacaaccaattaaccaattctgattagaaaaactcatcgagcatcaaatgaaactgcaatttattcatatcaggattatcaataccatatttttgaaaaagccgtttctgtaatgaaggagaaaactcaccgaggcagttccataggatggcaagatcctggtatcggtctgcgattccgactcgtccaacatcaatacaacctattaatttcccctcgtcaaaaataaggttatcaagtgagaaatcaccatgagtgacgactgaatccggtgagaatggcaaaagtttatgcatttctttccagacttgttcaacaggccagccattacgctcgtcatcaaaatcactcgcatcaaccaaaccgttattcattcgtgattgcgcctgagcgagacgaaatacgcgatcgctgttaaaaggacaattacaaacaggaatcgaatgcaaccggcgcagggacactgccagcgcatcaacaatattttcacctgaatcaggatattcttctaatacctggaatgctgtttttccggggatcgcagtggtgagtaaccatgcatcatcaggagtacggataaaatgcttgatggtcggaagaggcataaattccgtcagccagtttagtctgaccatctcatctgtaacatcattggcaacgctacctttgccatgtttcagaaacaactctggcgcatcgggcttcccatacaagcgatagattgtcgcacctgattgcccgacattatcgcgagcccatttatacccatataaatcagcatccatgttggaatttaatcgcggcctcgacgtttcccgttgaatatggctcataacaccccttgtattactgtttatgtaagcagacagttttattgttcatgatgatatatttttatcttgtgcaatgtaacatcagagattttgagacacgggccagagctgcagtttgatcccgaggggaaccctgtggttgacatgcacatacaaatggacgaacggataaaccttttcacgcccttttaaatatccgttattctaataaa

SEQ ID NO: 56 - DNA, 23 bp, synthetic construct
  source 1..23: mol_type = other DNA
cacttacttctcttcagttttcc

SEQ ID NO: 57 - DNA, 22 bp, synthetic construct
  source 1..22: mol_type = other DNA
atagtatcaatccagctcaatt

SEQ ID NO: 58 - DNA, 21 bp, synthetic construct
  source 1..21: mol_type = other DNA
ctacgttggaccacttgctag

SEQ ID NO: 59 - DNA, 22 bp, synthetic construct
  source 1..22: mol_type = other DNA
ctctcgatgaaagactgagcag

SEQ ID NO: 60 - DNA, 20 bp, synthetic construct
  source 1..20: mol_type = other DNA
gtgcgttatggctccactag

SEQ ID NO: 61 - DNA, 22 bp, synthetic construct
  source 1..22: mol_type = other DNA
gttctccagcatcacatttctg

SEQ ID NO: 62 - DNA, 20 bp, synthetic construct
  source 1..20: mol_type = other DNA
ccattccaattttcgccacg

SEQ ID NO: 63 - DNA, 21 bp, synthetic construct
  source 1..21: mol_type = other DNA
taccaaatcagcgtccatagg

SEQ ID NO: 64 - DNA, 20 bp, synthetic construct
  source 1..20: mol_type = other DNA
tatcggcggagagatttgag

SEQ ID NO: 65 - DNA, 20 bp, synthetic construct
  source 1..20: mol_type = other DNA
taagcccttcccttgattcc

SEQ ID NO: 66 - DNA, 20 bp, synthetic construct
  source 1..20: mol_type = other DNA
atgagaaactatggcctcgc

SEQ ID NO: 67 - DNA, 21 bp, synthetic construct
  source 1..21: mol_type = other DNA
agtagactttgggacagcaac

SEQ ID NO: 68 - DNA, 20 bp, synthetic construct
  source 1..20: mol_type = other DNA
tgacgtaagggatgacgcac

SEQ ID NO: 69 - DNA, 20 bp, synthetic construct
  source 1..20: mol_type = other DNA
gtcctttcccgtagtccagc

SEQ ID NO: 70 - DNA, 20 bp, synthetic construct
  source 1..20: mol_type = other DNA
atgttggggtcagacgcttt

SEQ ID NO: 71 - DNA, 20 bp, synthetic construct
  source 1..20: mol_type = other DNA
agaccggcaacaggattcaa

SEQ ID NO: 72 - DNA, 20 bp, synthetic construct
  source 1..20: mol_type = other DNA
gagcatcccacggagaaaca

SEQ ID NO: 73 - DNA, 20 bp, synthetic construct
  source 1..20: mol_type = other DNA
agaccggcaacaggattcaa